European Patent Application EP 4 786 494 A1, published August 5, 2026. Title: 抗FGFR2 抗体和包含其的多特异性结合分子. Applicant: 南京维立志博生物科技股份有限公司. The sequence listing filed with the application follows.

SEQUENCE LISTING (117 sequences)

SEQ ID NO: 1 - protein, 449 aa, synthetic construct
QVTLKESGPGILQSSQTLSLTCSFSGFSLSTSGMGVSWIRQPSGKGLEWLAHIYWDNDKRYNPSLKSRLTISKDTSRNQVFLKITSVDTADTATYYCTRSDSSGSFDYWGQGTTLTVSSASTKGPSVFPLAPSSKSTSGGTAALGCLVKDYFPEPVTVSWNSGALTSGVHTFPAVLQSSGLYSLSSVVTVPSSSLGTQTYICNVNHKPSNTKVDKKVEPKSCDKTHTCPPCPAPELLGGPSVFLFPPKPKDTLMISRTPEVTCVVVDVSHEDPEVKFNWYVDGVEVHNAKTKPREEQYNSTYRVVSVLTVLHQDWLNGKEYKCKVSNKALPAPIEKTISKAKGQPREPQVYTLPPSRDELTKNQVSLTCLVKGFYPSDIAVEWESNGQPENNYKTTPPVLDSDGSFFLYSKLTVDKSRWQQGNVFSCSVMHEALHNHYTQKSLSLSPGK

SEQ ID NO: 2 - protein, 119 aa, synthetic construct
QVTLKESGPGILQSSQTLSLTCSFSGFSLSTSGMGVSWIRQPSGKGLEWLAHIYWDNDKRYNPSLKSRLTISKDTSRNQVFLKITSVDTADTATYYCTRSDSSGSFDYWGQGTTLTVSS

SEQ ID NO: 3 - protein, 7 aa, synthetic construct
TSGMGVS

SEQ ID NO: 4 - protein, 16 aa, synthetic construct
HIYWDNDKRYNPSLKS

SEQ ID NO: 5 - protein, 9 aa, synthetic construct
SDSSGSFDY

SEQ ID NO: 6 - protein, 214 aa, synthetic construct
DIQMTQTTSSLSASLGDRVTISCRASQDISNYLNWYQQKPDGTVKFLIYYTSTLHSGVPSRFSGSGSGTDYSLTISNLEQEDIATYFCQQGNTLPWTFGGGTKLEIKRTVAAPSVFIFPPSDEQLKSGTASVVCLLNNFYPREAKVQWKVDNALQSGNSQESVTEQDSKDSTYSLSSTLTLSKADYEKHKVYACEVTHQGLSSPVTKSFNRGEC

SEQ ID NO: 7 - protein, 107 aa, synthetic construct
DIQMTQTTSSLSASLGDRVTISCRASQDISNYLNWYQQKPDGTVKFLIYYTSTLHSGVPSRFSGSGSGTDYSLTISNLEQEDIATYFCQQGNTLPWTFGGGTKLEIK

SEQ ID NO: 8 - protein, 11 aa, synthetic construct
RASQDISNYLN

SEQ ID NO: 9 - protein, 7 aa, synthetic construct
YTSTLHS

SEQ ID NO: 10 - protein, 9 aa, synthetic construct
QQGNTLPWT

SEQ ID NO: 11 - protein, 451 aa, synthetic construct
QVQLKQSGPGLVQPSQSLSITCTVSGFSLTNYGVHWVRQSPGKGLEWLGVIWSDGSTDYDAAFISRLSISTDNSKSQVFFKMNSLQAADTAIYYCARKGDYDYDNYAMDYWGQGTSVTVSSASTKGPSVFPLAPSSKSTSGGTAALGCLVKDYFPEPVTVSWNSGALTSGVHTFPAVLQSSGLYSLSSVVTVPSSSLGTQTYICNVNHKPSNTKVDKKVEPKSCDKTHTCPPCPAPELLGGPSVFLFPPKPKDTLMISRTPEVTCVVVDVSHEDPEVKFNWYVDGVEVHNAKTKPREEQYNSTYRVVSVLTVLHQDWLNGKEYKCKVSNKALPAPIEKTISKAKGQPREPQVYTLPPSRDELTKNQVSLTCLVKGFYPSDIAVEWESNGQPENNYKTTPPVLDSDGSFFLYSKLTVDKSRWQQGNVFSCSVMHEALHNHYTQKSLSLSPGK

SEQ ID NO: 12 - protein, 121 aa, synthetic construct
QVQLKQSGPGLVQPSQSLSITCTVSGFSLTNYGVHWVRQSPGKGLEWLGVIWSDGSTDYDAAFISRLSISTDNSKSQVFFKMNSLQAADTAIYYCARKGDYDYDNYAMDYWGQGTSVTVSS

SEQ ID NO: 13 - protein, 5 aa, synthetic construct
NYGVH

SEQ ID NO: 14 - protein, 16 aa, synthetic construct
VIWSDGSTDYDAAFIS

SEQ ID NO: 15 - protein, 13 aa, synthetic construct
KGDYDYDNYAMDY

SEQ ID NO: 16 - protein, 214 aa, synthetic construct
DVVITQSPATLSVTPGDSVSLSCRASQSISNNLHWYQQKSHESPRLLIKYASQSISGIPSRFSGSGSGTDFTLSINSVETEDFGMYFCQQSNSWPLTFGAGTKLELKRTVAAPSVFIFPPSDEQLKSGTASVVCLLNNFYPREAKVQWKVDNALQSGNSQESVTEQDSKDSTYSLSSTLTLSKADYEKHKVYACEVTHQGLSSPVTKSFNRGEC

SEQ ID NO: 17 - protein, 107 aa, synthetic construct
DVVITQSPATLSVTPGDSVSLSCRASQSISNNLHWYQQKSHESPRLLIKYASQSISGIPSRFSGSGSGTDFTLSINSVETEDFGMYFCQQSNSWPLTFGAGTKLELK

SEQ ID NO: 18 - protein, 11 aa, synthetic construct
RASQSISNNLH

SEQ ID NO: 19 - protein, 7 aa, synthetic construct
YASQSIS

SEQ ID NO: 20 - protein, 9 aa, synthetic construct
QQSNSWPLT

SEQ ID NO: 21 - protein, 448 aa, synthetic construct
EVQLQQSGPELVKPGASVKIPCKASGYTFTDYNMDWVKQSHGKSLEWIGDINPKNGETFYNQKFKGKATLTVDRSSSTAYMELRSLTSEDTAVYFCAKRDLNWYFDYWGQGTTLTVSSASTKGPSVFPLAPSSKSTSGGTAALGCLVKDYFPEPVTVSWNSGALTSGVHTFPAVLQSSGLYSLSSVVTVPSSSLGTQTYICNVNHKPSNTKVDKKVEPKSCDKTHTCPPCPAPELLGGPSVFLFPPKPKDTLMISRTPEVTCVVVDVSHEDPEVKFNWYVDGVEVHNAKTKPREEQYNSTYRVVSVLTVLHQDWLNGKEYKCKVSNKALPAPIEKTISKAKGQPREPQVYTLPPSRDELTKNQVSLTCLVKGFYPSDIAVEWESNGQPENNYKTTPPVLDSDGSFFLYSKLTVDKSRWQQGNVFSCSVMHEALHNHYTQKSLSLSPGK

SEQ ID NO: 22 - protein, 118 aa, synthetic construct
EVQLQQSGPELVKPGASVKIPCKASGYTFTDYNMDWVKQSHGKSLEWIGDINPKNGETFYNQKFKGKATLTVDRSSSTAYMELRSLTSEDTAVYFCAKRDLNWYFDYWGQGTTLTVSS

SEQ ID NO: 23 - protein, 5 aa, synthetic construct
DYNMD

SEQ ID NO: 24 - protein, 17 aa, synthetic construct
DINPKNGETFYNQKFKG

SEQ ID NO: 25 - protein, 9 aa, synthetic construct
RDLNWYFDY

SEQ ID NO: 26 - protein, 447 aa, synthetic construct
QVQLQQSGAELARPGASVKLSCKASGYTFTNYGISWVKQRTGQGLEWIGEIYPRSGNTYYNEKFKGKATLTADKSSSTAYMELRSLTSEDSAVYFCARGDYSNSDYWGQGTTLTVSSASTKGPSVFPLAPSSKSTSGGTAALGCLVKDYFPEPVTVSWNSGALTSGVHTFPAVLQSSGLYSLSSVVTVPSSSLGTQTYICNVNHKPSNTKVDKKVEPKSCDKTHTCPPCPAPELLGGPSVFLFPPKPKDTLMISRTPEVTCVVVDVSHEDPEVKFNWYVDGVEVHNAKTKPREEQYNSTYRVVSVLTVLHQDWLNGKEYKCKVSNKALPAPIEKTISKAKGQPREPQVYTLPPSRDELTKNQVSLTCLVKGFYPSDIAVEWESNGQPENNYKTTPPVLDSDGSFFLYSKLTVDKSRWQQGNVFSCSVMHEALHNHYTQKSLSLSPGK

SEQ ID NO: 27 - protein, 117 aa, synthetic construct
QVQLQQSGAELARPGASVKLSCKASGYTFTNYGISWVKQRTGQGLEWIGEIYPRSGNTYYNEKFKGKATLTADKSSSTAYMELRSLTSEDSAVYFCARGDYSNSDYWGQGTTLTVSS

SEQ ID NO: 28 - protein, 5 aa, synthetic construct
NYGIS

SEQ ID NO: 29 - protein, 17 aa, synthetic construct
EIYPRSGNTYYNEKFKG

SEQ ID NO: 30 - protein, 8 aa, synthetic construct
GDYSNSDY

SEQ ID NO: 31 - protein, 214 aa, synthetic construct
DIQMTQTTSSLSASLGDRVTISCRASQDITDHLNWYQQKPDGTVKLLIYYTSRLHSGVPSRFSGSGSGTDYSLTISNLEQEDIATYFCQQGNTLPRTFGGGTKLEIKRTVAAPSVFIFPPSDEQLKSGTASVVCLLNNFYPREAKVQWKVDNALQSGNSQESVTEQDSKDSTYSLSSTLTLSKADYEKHKVYACEVTHQGLSSPVTKSFNRGEC

SEQ ID NO: 32 - protein, 107 aa, synthetic construct
DIQMTQTTSSLSASLGDRVTISCRASQDITDHLNWYQQKPDGTVKLLIYYTSRLHSGVPSRFSGSGSGTDYSLTISNLEQEDIATYFCQQGNTLPRTFGGGTKLEIK

SEQ ID NO: 33 - protein, 11 aa, synthetic construct
RASQDITDHLN

SEQ ID NO: 34 - protein, 7 aa, synthetic construct
YTSRLHS

SEQ ID NO: 35 - protein, 9 aa, synthetic construct
QQGNTLPRT

SEQ ID NO: 36 - protein, 449 aa, synthetic construct
QVTLKESGPGILQSSQTLSLTCSFSGFSLTTSGMGVSWIRQPSGKGLEWLAHIYWDDDKRYNPSLKSRLTISKDTSRNQVFLKITSVDTADTATYYCAGCDSSGSFDYWGQGTTLTVSSASTKGPSVFPLAPSSKSTSGGTAALGCLVKDYFPEPVTVSWNSGALTSGVHTFPAVLQSSGLYSLSSVVTVPSSSLGTQTYICNVNHKPSNTKVDKKVEPKSCDKTHTCPPCPAPELLGGPSVFLFPPKPKDTLMISRTPEVTCVVVDVSHEDPEVKFNWYVDGVEVHNAKTKPREEQYNSTYRVVSVLTVLHQDWLNGKEYKCKVSNKALPAPIEKTISKAKGQPREPQVYTLPPSRDELTKNQVSLTCLVKGFYPSDIAVEWESNGQPENNYKTTPPVLDSDGSFFLYSKLTVDKSRWQQGNVFSCSVMHEALHNHYTQKSLSLSPGK

SEQ ID NO: 37 - protein, 119 aa, synthetic construct
QVTLKESGPGILQSSQTLSLTCSFSGFSLTTSGMGVSWIRQPSGKGLEWLAHIYWDDDKRYNPSLKSRLTISKDTSRNQVFLKITSVDTADTATYYCAGCDSSGSFDYWGQGTTLTVSS

SEQ ID NO: 38 - protein, 16 aa, synthetic construct
HIYWDDDKRYNPSLKS

SEQ ID NO: 39 - protein, 9 aa, synthetic construct
CDSSGSFDY

SEQ ID NO: 40 - protein, 214 aa, synthetic construct
DIQMTQTTSSLSASLGDRVTITCRASQDISNYLNWYQQKPDGTVKLLIYYRSRLHSGVPSRFSGSGSGPEYSLTISNLEQEDIATYFCQQGNTLPWTFGGGTKLEIKRTVAAPSVFIFPPSDEQLKSGTASVVCLLNNFYPREAKVQWKVDNALQSGNSQESVTEQDSKDSTYSLSSTLTLSKADYEKHKVYACEVTHQGLSSPVTKSFNRGEC

SEQ ID NO: 41 - protein, 107 aa, synthetic construct
DIQMTQTTSSLSASLGDRVTITCRASQDISNYLNWYQQKPDGTVKLLIYYRSRLHSGVPSRFSGSGSGPEYSLTISNLEQEDIATYFCQQGNTLPWTFGGGTKLEIK

SEQ ID NO: 42 - protein, 7 aa, synthetic construct
YRSRLHS

SEQ ID NO: 43 - protein, 449 aa, synthetic construct
EVQLQQSGAELVRPGASVKLSCTASGFNIKDYYMHWVKQRPEQGLEWIGRIDPEDGDTEYAPKFQGKATMTADTSSNTAYLQLSSLTSEDTAVYYCTTYYYVSTYEDYWGQGTTLTVSSASTKGPSVFPLAPSSKSTSGGTAALGCLVKDYFPEPVTVSWNSGALTSGVHTFPAVLQSSGLYSLSSVVTVPSSSLGTQTYICNVNHKPSNTKVDKKVEPKSCDKTHTCPPCPAPELLGGPSVFLFPPKPKDTLMISRTPEVTCVVVDVSHEDPEVKFNWYVDGVEVHNAKTKPREEQYNSTYRVVSVLTVLHQDWLNGKEYKCKVSNKALPAPIEKTISKAKGQPREPQVYTLPPSRDELTKNQVSLTCLVKGFYPSDIAVEWESNGQPENNYKTTPPVLDSDGSFFLYSKLTVDKSRWQQGNVFSCSVMHEALHNHYTQKSLSLSPGK

SEQ ID NO: 44 - protein, 119 aa, synthetic construct
EVQLQQSGAELVRPGASVKLSCTASGFNIKDYYMHWVKQRPEQGLEWIGRIDPEDGDTEYAPKFQGKATMTADTSSNTAYLQLSSLTSEDTAVYYCTTYYYVSTYEDYWGQGTTLTVSS

SEQ ID NO: 45 - protein, 8 aa, synthetic construct
GFNIKDYY

SEQ ID NO: 46 - protein, 8 aa, synthetic construct
IDPEDGDT

SEQ ID NO: 47 - protein, 12 aa, synthetic construct
TTYYYVSTYEDY

SEQ ID NO: 48 - protein, 211 aa, synthetic construct
QIVLTQSPAIMSASLGEEITLTCSASSSVSHMHWYQQKSGTSPKLLIYSTSNLASGVPSRFSGSGSGTFYSLTISSVEAEDAADYYCHHWSSWTFGGGTKLEIKRTVAAPSVFIFPPSDEQLKSGTASVVCLLNNFYPREAKVQWKVDNALQSGNSQESVTEQDSKDSTYSLSSTLTLSKADYEKHKVYACEVTHQGLSSPVTKSFNRGEC

SEQ ID NO: 49 - protein, 104 aa, synthetic construct
QIVLTQSPAIMSASLGEEITLTCSASSSVSHMHWYQQKSGTSPKLLIYSTSNLASGVPSRFSGSGSGTFYSLTISSVEAEDAADYYCHHWSSWTFGGGTKLEIK

SEQ ID NO: 50 - protein, 10 aa, synthetic construct
SASSSVSHMH

SEQ ID NO: 51 - protein, 7 aa, synthetic construct
STSNLAS

SEQ ID NO: 52 - protein, 7 aa, synthetic construct
HHWSSWT

SEQ ID NO: 53 - protein, 451 aa, synthetic construct
QVTLKESGPGILQSSQTLSLTCSFSGFSLSTSGMGVSWIRQPSGKGLEWLAHIYWDDDKRYNSSLKSRLTISKDTSRNQVFLKITSVDTADTATYYCARSSDWDDYTMAYWGQGTSVTVSSASTKGPSVFPLAPSSKSTSGGTAALGCLVKDYFPEPVTVSWNSGALTSGVHTFPAVLQSSGLYSLSSVVTVPSSSLGTQTYICNVNHKPSNTKVDKKVEPKSCDKTHTCPPCPAPELLGGPSVFLFPPKPKDTLMISRTPEVTCVVVDVSHEDPEVKFNWYVDGVEVHNAKTKPREEQYNSTYRVVSVLTVLHQDWLNGKEYKCKVSNKALPAPIEKTISKAKGQPREPQVYTLPPSRDELTKNQVSLTCLVKGFYPSDIAVEWESNGQPENNYKTTPPVLDSDGSFFLYSKLTVDKSRWQQGNVFSCSVMHEALHNHYTQKSLSLSPGK

SEQ ID NO: 54 - protein, 121 aa, synthetic construct
QVTLKESGPGILQSSQTLSLTCSFSGFSLSTSGMGVSWIRQPSGKGLEWLAHIYWDDDKRYNSSLKSRLTISKDTSRNQVFLKITSVDTADTATYYCARSSDWDDYTMAYWGQGTSVTVSS

SEQ ID NO: 55 - protein, 16 aa, synthetic construct
HIYWDDDKRYNSSLKS

SEQ ID NO: 56 - protein, 11 aa, synthetic construct
SSDWDDYTMAY

SEQ ID NO: 57 - protein, 218 aa, synthetic construct
DIVLTQSPASLAVSLGQRATISCRASESIDDFGISFMHWYQQKPGQPPKLLIYRASNLESGIPARFSGSGSRADFTLTINPVETDDVATYYCQQSNKDPPTFGAGTNLELKRTVAAPSVFIFPPSDEQLKSGTASVVCLLNNFYPREAKVQWKVDNALQSGNSQESVTEQDSKDSTYSLSSTLTLSKADYEKHKVYACEVTHQGLSSPVTKSFNRGEC

SEQ ID NO: 58 - protein, 111 aa, synthetic construct
DIVLTQSPASLAVSLGQRATISCRASESIDDFGISFMHWYQQKPGQPPKLLIYRASNLESGIPARFSGSGSRADFTLTINPVETDDVATYYCQQSNKDPPTFGAGTNLELK

SEQ ID NO: 59 - protein, 15 aa, synthetic construct
RASESIDDFGISFMH

SEQ ID NO: 60 - protein, 7 aa, synthetic construct
RASNLES

SEQ ID NO: 61 - protein, 9 aa, synthetic construct
QQSNKDPPT

SEQ ID NO: 62 - protein, 448 aa, synthetic construct
EVQLQQSGPELVKPGASVKIPCKASGYTFTDYNMDWVKQSHGKSLEWIGDINPKNGETFYNQKFKGKATLTVDRSSNTAYMELRSLTSEDTAVYFCAKRDLNWYFDYWGQGTTLTVSSASTKGPSVFPLAPSSKSTSGGTAALGCLVKDYFPEPVTVSWNSGALTSGVHTFPAVLQSSGLYSLSSVVTVPSSSLGTQTYICNVNHKPSNTKVDKKVEPKSCDKTHTCPPCPAPELLGGPSVFLFPPKPKDTLMISRTPEVTCVVVDVSHEDPEVKFNWYVDGVEVHNAKTKPREEQYNSTYRVVSVLTVLHQDWLNGKEYKCKVSNKALPAPIEKTISKAKGQPREPQVYTLPPSRDELTKNQVSLTCLVKGFYPSDIAVEWESNGQPENNYKTTPPVLDSDGSFFLYSKLTVDKSRWQQGNVFSCSVMHEALHNHYTQKSLSLSPGK

SEQ ID NO: 63 - protein, 118 aa, synthetic construct
EVQLQQSGPELVKPGASVKIPCKASGYTFTDYNMDWVKQSHGKSLEWIGDINPKNGETFYNQKFKGKATLTVDRSSNTAYMELRSLTSEDTAVYFCAKRDLNWYFDYWGQGTTLTVSS

SEQ ID NO: 64 - protein, 8 aa, synthetic construct
GYTFTDYN

SEQ ID NO: 65 - protein, 8 aa, synthetic construct
INPKNGET

SEQ ID NO: 66 - protein, 8 aa, synthetic construct
INPKNEET

SEQ ID NO: 67 - protein, 11 aa, synthetic construct
AKRDLNWYFDY

SEQ ID NO: 68 - protein, 448 aa, synthetic construct
EVQLVQSGAEVKKPGATVKISCKASGYTFTDYNMDWVQQAPGKGLEWIGDINPKNGETFYAEKFQGRVTLTVDRSTNTAYMELSSLRSEDTAVYFCAKRDLNWYFDYWGQGTTVTVSSASTKGPSVFPLAPSSKSTSGGTAALGCLVKDYFPEPVTVSWNSGALTSGVHTFPAVLQSSGLYSLSSVVTVPSSSLGTQTYICNVNHKPSNTKVDKKVEPKSCDKTHTCPPCPAPELLGGPSVFLFPPKPKDTLMISRTPEVTCVVVDVSHEDPEVKFNWYVDGVEVHNAKTKPREEQYNSTYRVVSVLTVLHQDWLNGKEYKCKVSNKALPAPIEKTISKAKGQPREPQVYTLPPSRDELTKNQVSLTCLVKGFYPSDIAVEWESNGQPENNYKTTPPVLDSDGSFFLYSKLTVDKSRWQQGNVFSCSVMHEALHNHYTQKSLSLSPGK

SEQ ID NO: 69 - protein, 118 aa, synthetic construct
EVQLVQSGAEVKKPGATVKISCKASGYTFTDYNMDWVQQAPGKGLEWIGDINPKNGETFYAEKFQGRVTLTVDRSTNTAYMELSSLRSEDTAVYFCAKRDLNWYFDYWGQGTTVTVSS

SEQ ID NO: 70 - protein, 448 aa, synthetic construct
EVQLVQSGAEVKKPGATVKISCKASGYTFTDYNMDWVQQAPGKGLEWIGDINPKNGETFYAEKFQGRVTLTVDRSTNTAYMELSSLRSEDTAVYYCAKRDLNWYFDYWGQGTTVTVSSASTKGPSVFPLAPSSKSTSGGTAALGCLVKDYFPEPVTVSWNSGALTSGVHTFPAVLQSSGLYSLSSVVTVPSSSLGTQTYICNVNHKPSNTKVDKKVEPKSCDKTHTCPPCPAPELLGGPSVFLFPPKPKDTLMISRTPEVTCVVVDVSHEDPEVKFNWYVDGVEVHNAKTKPREEQYNSTYRVVSVLTVLHQDWLNGKEYKCKVSNKALPAPIEKTISKAKGQPREPQVYTLPPSRDELTKNQVSLTCLVKGFYPSDIAVEWESNGQPENNYKTTPPVLDSDGSFFLYSKLTVDKSRWQQGNVFSCSVMHEALHNHYTQKSLSLSPGK

SEQ ID NO: 71 - protein, 118 aa, synthetic construct
EVQLVQSGAEVKKPGATVKISCKASGYTFTDYNMDWVQQAPGKGLEWIGDINPKNGETFYAEKFQGRVTLTVDRSTNTAYMELSSLRSEDTAVYYCAKRDLNWYFDYWGQGTTVTVSS

SEQ ID NO: 72 - protein, 448 aa, synthetic construct
EVQLVQSGAEVKKPGATVKISCKASGYTFTDYNMDWVQQAPGKGLEWMGDINPKNGETFYAEKFQGRVTLTVDRSTNTAYMELSSLRSEDTAVYFCAKRDLNWYFDYWGQGTTVTVSSASTKGPSVFPLAPSSKSTSGGTAALGCLVKDYFPEPVTVSWNSGALTSGVHTFPAVLQSSGLYSLSSVVTVPSSSLGTQTYICNVNHKPSNTKVDKKVEPKSCDKTHTCPPCPAPELLGGPSVFLFPPKPKDTLMISRTPEVTCVVVDVSHEDPEVKFNWYVDGVEVHNAKTKPREEQYNSTYRVVSVLTVLHQDWLNGKEYKCKVSNKALPAPIEKTISKAKGQPREPQVYTLPPSRDELTKNQVSLTCLVKGFYPSDIAVEWESNGQPENNYKTTPPVLDSDGSFFLYSKLTVDKSRWQQGNVFSCSVMHEALHNHYTQKSLSLSPGK

SEQ ID NO: 73 - protein, 118 aa, synthetic construct
EVQLVQSGAEVKKPGATVKISCKASGYTFTDYNMDWVQQAPGKGLEWMGDINPKNGETFYAEKFQGRVTLTVDRSTNTAYMELSSLRSEDTAVYFCAKRDLNWYFDYWGQGTTVTVSS

SEQ ID NO: 74 - protein, 448 aa, synthetic construct
EVQLVQSGAEVKKPGATVKISCKASGYTFTDYNMDWVQQAPGKGLEWMGDINPKNEETFYAEKFQGRVTLTVDRSTNTAYMELSSLRSEDTAVYFCAKRDLNWYFDYWGQGTTVTVSSASTKGPSVFPLAPSSKSTSGGTAALGCLVKDYFPEPVTVSWNSGALTSGVHTFPAVLQSSGLYSLSSVVTVPSSSLGTQTYICNVNHKPSNTKVDKKVEPKSCDKTHTCPPCPAPELLGGPSVFLFPPKPKDTLMISRTPEVTCVVVDVSHEDPEVKFNWYVDGVEVHNAKTKPREEQYNSTYRVVSVLTVLHQDWLNGKEYKCKVSNKALPAPIEKTISKAKGQPREPQVYTLPPSRDELTKNQVSLTCLVKGFYPSDIAVEWESNGQPENNYKTTPPVLDSDGSFFLYSKLTVDKSRWQQGNVFSCSVMHEALHNHYTQKSLSLSPGK

SEQ ID NO: 75 - protein, 118 aa, synthetic construct
EVQLVQSGAEVKKPGATVKISCKASGYTFTDYNMDWVQQAPGKGLEWMGDINPKNEETFYAEKFQGRVTLTVDRSTNTAYMELSSLRSEDTAVYFCAKRDLNWYFDYWGQGTTVTVSS

SEQ ID NO: 76 - protein, 448 aa, synthetic construct
EVQLVQSGAEVKKPGASVKVSCKASGYTFTDYNMDWVRQAPGQRLEWMGDINPKNGETFYSQKFQGRVTITVDTSASTAYMELSSLRSEDTAVYYCAKRDLNWYFDYWGQGTTVTVSSASTKGPSVFPLAPSSKSTSGGTAALGCLVKDYFPEPVTVSWNSGALTSGVHTFPAVLQSSGLYSLSSVVTVPSSSLGTQTYICNVNHKPSNTKVDKKVEPKSCDKTHTCPPCPAPELLGGPSVFLFPPKPKDTLMISRTPEVTCVVVDVSHEDPEVKFNWYVDGVEVHNAKTKPREEQYNSTYRVVSVLTVLHQDWLNGKEYKCKVSNKALPAPIEKTISKAKGQPREPQVYTLPPSRDELTKNQVSLTCLVKGFYPSDIAVEWESNGQPENNYKTTPPVLDSDGSFFLYSKLTVDKSRWQQGNVFSCSVMHEALHNHYTQKSLSLSPGK

SEQ ID NO: 77 - protein, 118 aa, synthetic construct
EVQLVQSGAEVKKPGASVKVSCKASGYTFTDYNMDWVRQAPGQRLEWMGDINPKNGETFYSQKFQGRVTITVDTSASTAYMELSSLRSEDTAVYYCAKRDLNWYFDYWGQGTTVTVSS

SEQ ID NO: 78 - protein, 448 aa, synthetic construct
EVQLVQSGAEVKKPGASVKVSCKASGYTFTDYNMDWVRQAPGQRLEWMGDINPKNEETFYSQKFQGRVTITVDTSASTAYMELSSLRSEDTAVYYCAKRDLNWYFDYWGQGTTVTVSSASTKGPSVFPLAPSSKSTSGGTAALGCLVKDYFPEPVTVSWNSGALTSGVHTFPAVLQSSGLYSLSSVVTVPSSSLGTQTYICNVNHKPSNTKVDKKVEPKSCDKTHTCPPCPAPELLGGPSVFLFPPKPKDTLMISRTPEVTCVVVDVSHEDPEVKFNWYVDGVEVHNAKTKPREEQYNSTYRVVSVLTVLHQDWLNGKEYKCKVSNKALPAPIEKTISKAKGQPREPQVYTLPPSRDELTKNQVSLTCLVKGFYPSDIAVEWESNGQPENNYKTTPPVLDSDGSFFLYSKLTVDKSRWQQGNVFSCSVMHEALHNHYTQKSLSLSPGK

SEQ ID NO: 79 - protein, 118 aa, synthetic construct
EVQLVQSGAEVKKPGASVKVSCKASGYTFTDYNMDWVRQAPGQRLEWMGDINPKNEETFYSQKFQGRVTITVDTSASTAYMELSSLRSEDTAVYYCAKRDLNWYFDYWGQGTTVTVSS

SEQ ID NO: 80 - protein, 214 aa, synthetic construct
DIQMTQSSSYLSVSLGGRVTITCKASDHINNWLAWYQQKPGNAPRLLISGATSLETGVPSRFSGSGSGKDYTLSITSLQTEDVATYYCQQYWSTPWTFGGGTKLEIKRTVAAPSVFIFPPSDEQLKSGTASVVCLLNNFYPREAKVQWKVDNALQSGNSQESVTEQDSKDSTYSLSSTLTLSKADYEKHKVYACEVTHQGLSSPVTKSFNRGEC

SEQ ID NO: 81 - protein, 107 aa, synthetic construct
DIQMTQSSSYLSVSLGGRVTITCKASDHINNWLAWYQQKPGNAPRLLISGATSLETGVPSRFSGSGSGKDYTLSITSLQTEDVATYYCQQYWSTPWTFGGGTKLEIK

SEQ ID NO: 82 - protein, 6 aa, synthetic construct
DHINNW

SEQ ID NO: 83 - skipped

SEQ ID NO: 84 - protein, 9 aa, synthetic construct
QQYWSTPWT

SEQ ID NO: 85 - protein, 214 aa, synthetic construct
DIQMTQSPSSLSASVGDRVTITCQASDHINNWLAWYQQKPGKAPKLLISGATSLETGVPSRFSGSGSGKDYTFTISSLQPEDIATYYCQQYWSTPWTFGGGTKVEIKRTVAAPSVFIFPPSDEQLKSGTASVVCLLNNFYPREAKVQWKVDNALQSGNSQESVTEQDSKDSTYSLSSTLTLSKADYEKHKVYACEVTHQGLSSPVTKSFNRGEC

SEQ ID NO: 86 - protein, 107 aa, synthetic construct
DIQMTQSPSSLSASVGDRVTITCQASDHINNWLAWYQQKPGKAPKLLISGATSLETGVPSRFSGSGSGKDYTFTISSLQPEDIATYYCQQYWSTPWTFGGGTKVEIK

SEQ ID NO: 87 - protein, 214 aa, synthetic construct
DIQMTQSPSSLSASVGDRVTITCQASDHINNWLAWYQQKPGKAPKLLISGATSLETGVPSRFSGSGSGKDFTFTISSLQPEDIATYYCQQYWSTPWTFGGGTKVEIKRTVAAPSVFIFPPSDEQLKSGTASVVCLLNNFYPREAKVQWKVDNALQSGNSQESVTEQDSKDSTYSLSSTLTLSKADYEKHKVYACEVTHQGLSSPVTKSFNRGEC

SEQ ID NO: 88 - protein, 107 aa, synthetic construct
DIQMTQSPSSLSASVGDRVTITCQASDHINNWLAWYQQKPGKAPKLLISGATSLETGVPSRFSGSGSGKDFTFTISSLQPEDIATYYCQQYWSTPWTFGGGTKVEIK

SEQ ID NO: 89 - protein, 561 aa, synthetic construct
EVQLVQSGAEVKKPGATVKISCKASGYTFTDYNMDWVQQAPGKGLEWMGDINPKNGETFYAEKFQGRVTLTVDRSTNTAYMELSSLRSEDTAVYFCAKRDLNWYFDYWGQGTTVTVSSASTKGPSVFPLAPSSKSTSGGTAALGCLVKDYFPEPVTVSWNSGALTSGVHTFPAVLQSSGLYSLSSVVTVPSSSLGTQTYICNVNHKPSNTKVDKKVEPKSCDKTHTCPPCPAPELLGGPSVFLFPPKPKDTLMISRTPEVTCVVVDVSHEDPEVKFNWYVDGVEVHNAKTKPREEQYNSTYRVVSVLTVLHQDWLNGKEYKCKVSNKALPAPIEKTISKAKGQPREPQVYTLPPSRDELTKNQVSLTCLVKGFYPSDIAVEWESNGQPENNYKTTPPVLDSDGSFFLYSKLTVDKSRWQQGNVFSCSVMHEALHNHYTQKSLSLSPGAGGGGSGGGGSGGGGSGRPFVEMYSEIPEIIHMTEGRELVIPCRVTSPNITVTLKKFPLDTLIPDGKRIIWDSRKGFIISNATYKEIGLLTCEATVNGHLYKTNYLTHRQTNTI

SEQ ID NO: 90 - protein, 15 aa, synthetic construct
GGGGSGGGGSGGGGS

SEQ ID NO: 91 - protein, 330 aa, synthetic construct [sequence omitted]

SEQ ID NO: 92 - protein, 107 aa, synthetic construct [sequence omitted]

SEQ ID NO: 93 - protein, 227 aa, synthetic construct
DKTHTCPPCPAPELLGGPSVFLFPPKPKDTLMISRTPEVTCVVVDVSHEDPEVKFNWYVDGVEVHNAKTKPREEQYNSTYRVVSVLTVLHQDWLNGKEYKCKVSNKALPAPIEKTISKAKGQPREPQVYTLPPSRDELTKNQVSLTCLVKGFYPSDIAVEWESNGQPENNYKTTPPVLDSDGSFFLYSKLTVDKSRWQQGNVFSCSVMHEALHNHYTQKSLSLSPGK

SEQ ID NO: 94 - protein, 233 aa, synthetic construct
RAPYWTNTEKMEKRLHAVPAANTVKFRCPAGGNPMPTMRWLKNGKEFKQEHRIGGYKVRNQHWSLIMESVVPSDKGNYTCVVENEYGSINHTYHLDVVERSPHRPILQAGLPANASTVVGGDVEFVCKVYSDAQPHIQWIKHVEKNGSKYGPDGLPYLKVLKHSGINSSNAEVLALFNVTEADAGEYICKVSNYIGQANQSAWLTVLPKQQAPGREKEITASPDYLEHHHHHH

SEQ ID NO: 95 - protein, 233 aa, synthetic construct
RAPYWTNTEKMEKRLHAVPAANTVKFRCPAGGNPTPTMRWLKNGKEFKQEHRIGGYKVRNQHWSLIMESVVPSDKGNYTCVVENEYGSINHTYHLDVVERSPHRPILQAGLPANASTVVGGDVEFVCKVYSDAQPHIQWIKHVEKNGSKYGPDGLPYLKVLKHSGINSSNAEVLALFNVTEADAGEYICKVSNYIGQANQSAWLTVLPKQQAPGREKEITASPDYLEHHHHHH

SEQ ID NO: 96 - protein, 103 aa, synthetic construct
ASTKGPSVFPLAPSSKSTSGGTAALGCLVKDYFPEPVTVSWNSGALTSGVHTFPAVLQSSGLYSLSSVVTVPSSSLGTQTYICNVNHKPSNTKVDKKVEPKSC

SEQ ID NO: 97 - protein, 227 aa, synthetic construct
DKTHTCPPCPAPELLGGPSVFLFPPKPKDTLMISRTPEVTCVVVDVSHEDPEVKFNWYVDGVEVHNAKTKPREEQYNSTYRVVSVLTVLHQDWLNGKEYKCKVSNKALPAPIEKTISKAKGQPREPQVYTLPPSRDELTKNQVSLTCLVKGFYPSDIAVEWESNGQPENNYKTTPPVLDSDGSFFLYSKLTVDKSRWQQGNVFSCSVMHEALHNHYTQKSLSLSPGA

SEQ ID NO: 98 - protein, 444 aa, synthetic construct
QVQLVQSGAEVKKPGSSVKVSCKASGYIFTTYNVHWVRQAPGQGLEWIGSIYPDNGDTSYNQNFKGRATITADKSTSTAYMELSSLRSEDTAVYYCARGDFAYWGQGTLVTVSSASTKGPSVFPLAPSSKSTSGGTAALGCLVKDYFPEPVTVSWNSGALTSGVHTFPAVLQSSGLYSLSSVVTVPSSSLGTQTYICNVNHKPSNTKVDKKVEPKSCDKTHTCPPCPAPELLGGPSVFLFPPKPKDTLMISRTPEVTCVVVDVSHEDPEVKFNWYVDGVEVHNAKTKPREEQYNSTYRVVSVLTVLHQDWLNGKEYKCKVSNKALPAPIEKTISKAKGQPREPQVYTLPPSRDELTKNQVSLTCLVKGFYPSDIAVEWESNGQPENNYKTTPPVLDSDGSFFLYSKLTVDKSRWQQGNVFSCSVMHEALHNHYTQKSLSLSPGK

SEQ ID NO: 99 - protein, 214 aa, synthetic construct
DIQMTQSPSSLSASVGDRVTITCKASQGVSNDVAWYQQKPGKAPKLLIYSASYRYTGVPSRFSGSGSGTDFTFTISSLQPEDIATYYCQQHSTTPYTFGQGTKLEIKRTVAAPSVFIFPPSDEQLKSGTASVVCLLNNFYPREAKVQWKVDNALQSGNSQESVTEQDSKDSTYSLSSTLTLSKADYEKHKVYACEVTHQGLSSPVTKSFNRGEC

SEQ ID NO: 100 - protein, 98 aa, synthetic construct
GRPFVEMYSEIPEIIHMTEGRELVIPCRVTSPNITVTLKKFPLDTLIPDGKRIIWDSRKGFIISNATYKEIGLLTCEATVNGHLYKTNYLTHRQTNTI

SEQ ID NO: 101 - protein, 1312 aa, synthetic construct
SKLKDPELSLKGTQHIMQAGQTLHLQCRGEAAHKWSLPEMVSKESERLSITKSACGRNGKQFCSTLTLNTAQANHTGFYSCKYLAVPTSKKKETESAIYIFISDTGRPFVEMYSEIPEIIHMTEGRELVIPCRVTSPNITVTLKKFPLDTLIPDGKRIIWDSRKGFIISNATYKEIGLLTCEATVNGHLYKTNYLTHRQTNTIIDVQISTPRPVKLLRGHTLVLNCTATTPLNTRVQMTWSYPDEKNKRASVRRRIDQSNSHANIFYSVLTIDKMQNKDKGLYTCRVRSGPSFKSVNTSVHIYDKAFITVKHRKQQVLETVAGKRSYRLSMKVKAFPSPEVVWLKDGLPATEKSARYLTRGYSLIIKDVTEEDAGNYTILLSIKQSNVFKNLTATLIVNVKPQIYEKAVSSFPDPALYPLGSRQILTCTAYGIPQPTIKWFWHPCNHNHSEARCDFCSNNEESFILDADSNMGNRIESITQRMAIIEGKNKMASTLVVADSRISGIYICIASNKVGTVGRNISFYITDVPNGFHVNLEKMPTEGEDLKLSCTVNKFLYRDVTWILLRTVNNRTMHYSISKQKMAITKEHSITLNLTIMNVSLQDSGTYACRARNVYTGEEILQKKEITIRDQEAPYLLRNLSDHTVAISSSTTLDCHANGVPEPQITWFKNNHKIQQEPGIILGPGSSTLFIERVTEEDEGVYHCKATNQKGSVESSAYLTVQGTSDKSNLELITLTCTCVAATLFWLLLTLFIRKMKRSSSEIKTDYLSIIMDPDEVPLDEQCERLPYDASKWEFARERLKLGKSLGRGAFGKVVQASAFGIKKSPTCRTVAVKMLKEGATASEYKALMTELKILTHIGHHLNVVNLLGACTKQGGPLMVIVEYCKYGNLSNYLKSKRDLFFLNKDAALHMEPKKEKMEPGLEQGKKPRLDSVTSSESFASSGFQEDKSLSDVEEEEDSDGFYKEPITMEDLISYSFQVARGMEFLSSRKCIHRDLAARNILLSENNVVKICDFGLARDIYKNPDYVRKGDTRLPLKWMAPESIFDKIYSTKSDVWSYGVLLWEIFSLGGSPYPGVQMDEDFCSRLREGMRMRAPEYSTPEIYQIMLDCWHRDPKERPRFAELVEKLGDLLQANVQQDGKDYIPINAILTGNSGFTYSTPAFSEDFFKESISAPKFNSGSSDDVRYVNAFKFMSLERIKTFEELLPNATSMFDDYQGDSSTLLASPMLKRFTWTDSKPKASLKIDLRVTSKSKESGLSDVSRPSFCHSSCGHVSEGKRRFTYDHAELERKIACCSPPPDYNSVVLYSTPPI

SEQ ID NO: 102 - protein, 732 aa, synthetic construct
SKLKDPELSLKGTQHIMQAGQTLHLQCRGEAAHKWSLPEMVSKESERLSITKSACGRNGKQFCSTLTLNTAQANHTGFYSCKYLAVPTSKKKETESAIYIFISDTGRPFVEMYSEIPEIIHMTEGRELVIPCRVTSPNITVTLKKFPLDTLIPDGKRIIWDSRKGFIISNATYKEIGLLTCEATVNGHLYKTNYLTHRQTNTIIDVQISTPRPVKLLRGHTLVLNCTATTPLNTRVQMTWSYPDEKNKRASVRRRIDQSNSHANIFYSVLTIDKMQNKDKGLYTCRVRSGPSFKSVNTSVHIYDKAFITVKHRKQQVLETVAGKRSYRLSMKVKAFPSPEVVWLKDGLPATEKSARYLTRGYSLIIKDVTEEDAGNYTILLSIKQSNVFKNLTATLIVNVKPQIYEKAVSSFPDPALYPLGSRQILTCTAYGIPQPTIKWFWHPCNHNHSEARCDFCSNNEESFILDADSNMGNRIESITQRMAIIEGKNKMASTLVVADSRISGIYICIASNKVGTVGRNISFYITDVPNGFHVNLEKMPTEGEDLKLSCTVNKFLYRDVTWILLRTVNNRTMHYSISKQKMAITKEHSITLNLTIMNVSLQDSGTYACRARNVYTGEEILQKKEITIRDQEAPYLLRNLSDHTVAISSSTTLDCHANGVPEPQITWFKNNHKIQQEPGIILGPGSSTLFIERVTEEDEGVYHCKATNQKGSVESSAYLTVQGTSDKSNLE

SEQ ID NO: 103 - protein, 274 aa, Homo sapiens [sequence omitted]

SEQ ID NO: 104 - protein, 119 aa, synthetic construct
EVQLVQSGAEVKKPGATVKISCKASGFNIKDYYMHWVQQAPGKGLEWMGRIDPEDGDTEYAEKFQGRVTITADTSTNTAYMELSSLRSEDTAVYYCTTYYYVSTYEDYWGQGTTVTVSS

SEQ ID NO: 105 - protein, 104 aa, synthetic construct
EIVLTQSPATLSLSPGERATLSCRASSSVSHMHWYQQKPGQAPKLLIYSTSNLASGVPARFSGSGSGTDYTLTISSLEPEDFAVYYCHHWSSWTFGGGTKVEIK

SEQ ID NO: 106 - protein, 449 aa, synthetic construct
EVQLVQSGAEVKKPGATVKISCKASGFNIKDYYMHWVQQAPGKGLEWMGRIDPEDGDTEYAEKFQGRVTITADTSTNTAYMELSSLRSEDTAVYYCTTYYYVSTYEDYWGQGTTVTVSSASTKGPSVFPLAPSSKSTSGGTAALGCLVKDYFPEPVTVSWNSGALTSGVHTFPAVLQSSGLYSLSSVVTVPSSSLGTQTYICNVNHKPSNTKVDKKVEPKSCDKTHTCPPCPAPELLGGPSVFLFPPKPKDTLMISRTPEVTCVVVDVSHEDPEVKFNWYVDGVEVHNAKTKPREEQYNSTYRVVSVLTVLHQDWLNGKEYKCKVSNKALPAPIEKTISKAKGQPREPQVYTLPPSRDELTKNQVSLTCLVKGFYPSDIAVEWESNGQPENNYKTTPPVLDSDGSFFLYSKLTVDKSRWQQGNVFSCSVMHEALHNHYTQKSLSLSPGK

SEQ ID NO: 107 - protein, 211 aa, synthetic construct
EIVLTQSPATLSLSPGERATLSCRASSSVSHMHWYQQKPGQAPKLLIYSTSNLASGVPARFSGSGSGTDYTLTISSLEPEDFAVYYCHHWSSWTFGGGTKVEIKRTVAAPSVFIFPPSDEQLKSGTASVVCLLNNFYPREAKVQWKVDNALQSGNSQESVTEQDSKDSTYSLSSTLTLSKADYEKHKVYACEVTHQGLSSPVTKSFNRGEC

SEQ ID NO: 108 - protein, 453 aa, synthetic construct
EVQLVESGGGLVQPGGSLRLSCAASGYTFTNYGMNWVRQAPGKGLEWVGWINTYTGEPTYAADFKRRFTFSLDTSKSTAYLQMNSLRAEDTAVYYCAKYPHYYGSSHWYFDVWGQGTLVTVSSASTKGPSVFPLAPSSKSTSGGTAALGCLVKDYFPEPVTVSWNSGALTSGVHTFPAVLQSSGLYSLSSVVTVPSSSLGTQTYICNVNHKPSNTKVDKKVEPKSCDKTHTCPPCPAPEAAGGPSVFLFPPKPKDTLMISRTPEVTCVVVAVSHEDPEVKFNWYVDGVEVHNAKTKPREEQYNSTYRVVSVLTVLHQDWLNGKEYKCKVSNKALAAPIEKTISKAKGQPREPQVYTLPPSRDELTKNQVSLTCLVKGFYPSDIAVEWESNGQPENNYKTTPPVLDSDGSFFLYSKLTVDKSRWQQGNVFSCSVMHEALHNHYTQKSLSLSPGK

SEQ ID NO: 109 - protein, 214 aa, synthetic construct
DIQMTQSPSSLSASVGDRVTITCSASQDISNYLNWYQQKPGKAPKVLIYFTSSLHSGVPSRFSGSGSGTDFTLTISSLQPEDFATYYCQQYSTVPWTFGQGTKVEIKRTVAAPSVFIFPPSDEQLKSGTASVVCLLNNFYPREAKVQWKVDNALQSGNSQESVTEQDSKDSTYSLSSTLTLSKADYEKHKVYACEVTHQGLSSPVTKSFNRGEC

SEQ ID NO: 110 - protein, 565 aa, synthetic construct
QMQLVQSGAEVKKPGASVKLSCKASGYPFQSYYIHWVRQAPGQGLEWVGVINPSGGSTTYAQKFQGRVTMTRDTSISTAYMELSRLRSDDTVVYYCARGSYSSGWDYYYYYGMDVWGKGTLVTVSSASTKGPSVFPLAPSSKSTSGGTAALGCLVKDYFPEPVTVSWNSGALTSGVHTFPAVLQSSGLYSLSSVVTVPSSSLGTQTYICNVNHKPSNTKVDKKVEPKSCDKTHTCPPCPAPEAAGGPSVFLFPPKPKDTLMISRTPEVTCVVVAVSHEDPEVKFNWYVDGVEVHNAKTKPREEQYNSTYRVVSVLTVLHQDWLNGKEYKCKVSNKALAAPIEKTISKAKGQPREPQVYTLPPSRDELTKNQVSLTCLVKGFYPSDIAVEWESNGQPENNYKTTPPVLDSDGSFFLYSKLTVDKSRWQQGNVFSCSVMHEALHNHYTQKSLSLSPGASPAPELLGGPSGRPFVEMYSEIPEIIHMTEGRELVIPCRVTSPNITVTLKKFPLDTLIPDGKRIIWDSRKGFIISNATYKEIGLLTCEATVNGHLYKTNYLTHRQTNTI

SEQ ID NO: 111 - protein, 219 aa, synthetic construct
DVVMTQSPLSLPVTPGEPASISCRSSQSLLHSQGYNYLDWYLQKPGQSPQLLIYLGSNRASGVPDRFSGSGSGTDFTLKISRVEAEDVGVYYCMQALQTPWTFGQGTKVEIKRTVAAPSVFIFPPSDEQLKSGTASVVCLLNNFYPREAKVQWKVDNALQSGNSQESVTEQDSKDSTYSLSSTLTLSKADYEKHKVYACEVTHQGLSSPVTKSFNRGEC

SEQ ID NO: 112-113 - skipped (2 entries)

SEQ ID NO: 114 - protein, 5 aa, synthetic construct
  REPEAT 1..5: note = Repeated for n times, wherein n is an integer equal to or more than 1, for exmaple, n is a integer selected from 2, 3, 4, 5, 6, 7, 8, 9, 10.
GSGGS

SEQ ID NO: 115 - protein, 5 aa, synthetic construct
  REPEAT 1..5: note = Repeated for n times, wherein n is an integer equal to or more than 1, for exmaple, n is a integer selected from 2, 3, 4, 5, 6, 7, 8, 9, 10.
GGGGS

SEQ ID NO: 116 - protein, 4 aa, synthetic construct
  REPEAT 1..4: note = Repeated for n times, wherein n is an integer equal to or more than 1, for exmaple, n is a integer selected from 2, 3, 4, 5, 6, 7, 8, 9, 10.
GGGS

SEQ ID NO: 117 - protein, 6 aa, synthetic construct
  REPEAT 1..5: note = Repeated for n times, wherein n is an integer equal to or more than 1, for exmaple, n is a integer selected from 2, 3, 4, 5, 6, 7, 8, 9, 10
GGGGSG